European Patent Specification EP 3 145 529 B1, published November 15, 2023. Title: TREATMENT OF MYOTONIC DYSTROPHY. Applicant: ASSOCIATION INSTITUT DE MYOLOGIE ET AL. The sequence listing filed with the application follows.

SEQUENCE LISTING (7 sequences)

SEQ ID NO: 1 - protein, 130 aa, homo sapiens
TQSAVKSLKRPLEATFDLGIPQAVLPPLPKRPALEKTNGATAVFNTGIFQYQQALANMQLQQHTAFLPPGSILCMTPATSVVPMVHGATPATVSAATTSATSVPFAATTANQIPIISAEHLTSHKYVTQM

SEQ ID NO: 2 - protein, 269 aa, artificial
  delta-CT3 MBNL1-derived polypeptide
MAVSVTPIRDTKWLTLEVCREFQRGTCSRPDTECKFAHPSKSCQVENGRVIACFDSLKGRCSRENCKYLHPPPHLKTQLEINGRNNLIQQKNMAMLAQQMQLANAMMPGAPLQPVPMFSVAPSLATNASAAAFNPYLGPVSPSLVPAEILPTAPMLVTGNPGVPVPAAAAAAAQKLMRTDRLEVCREYQRGNCNRGENDCRFAHPADSTMIDTNDNTVTVCMDYIKGRCSREKCKYFHPPAHLQAKIKAAQYQVNQAAAAQAAATAAAM

SEQ ID NO: 3 - protein, 201 aa, artificial
  delta-CT MBNL1-derived polypeptide
MAVSVTPIRDTKWLTLEVCREFQRGTCSRPDTECKFAHPSKSCQVENGRVIACFDSLKGRCSRENCKYLHPPPHLKTQLEINGRNNLIQQKNMAMLAQQMQLANAMMPGAPLQPVVCREYQRGNCNRGENDCRFAHPADSTMIDTNDNTVTVCMDYIKGRCSREKCKYFHPPAHLQAKIKAAQYQVNQAAAAQAAATAAAM

SEQ ID NO: 4 - protein, 268 aa, artificial
  delta-CT3 MBNL2-derived polypeptide
MALNVAPVRDTKWLTLEVCRQFQRGTCSRSDEECKFAHPPKSCQVENGRVIACFDSLKGRCSRENCKYLHPPTHLKTQLEINGRNNLIQQKTAAAMLAQQMQFMFPGTPLHPVPTFPVGPAIGTNTAISFAPYLAPVTPGVGLVPTEILPTTPVIVPGSPPVTVPGSTATQKLLRTDKLEVCREFQRGNCARGETDCRFAHPADSTMIDTSDNTVTVCMDYIKGRCMREKCKYFHPPAHLQAKIKAAQHQANQAAVAAQAAAAAATVM

SEQ ID NO: 5 - protein, 7 aa, artificial
  NLS
PKKKRKV

SEQ ID NO: 6 - protein, 10 aa, artificial
  NES
LPPLERLTLD

SEQ ID NO: 7 - DNA, 568 bp, artificial
  mutated MBNL minigene
cctttcacccaggagcaaacgcacatcacctgtgtcctcatctgatggccctggtgtggggcacagtcgtgttggcagggagggaggtggggttggtcccctttgtgggtttgttgcgaggccgtgttccagctgtttccacagggagcgattttcagctccacaggacacagctccccagttcctcctgagaacaaaagggggttctggggagaggccaccgttctgagggctcactgtatgtgttccagaatctcccctgcagacccccactgaggacggatctgaggaaccgggctctgaaacctctgaccgtaagagcactccaacagcggaaggtgggccccccttcagacgccccctccagcctccagcctgtacttagcctactttgagcctccctcctggctgcatctacgctccccctggctgagagatgtcactccttcggtactcaggacagcgtggtgggagctgagccttcgattacttactggttgagtgtgggcaccttcatcccgtgtggctctggaggcagccacccttggacagtcccgcgcacagctcc